European Patent Specification EP 3 728 571 B1, published September 17, 2025. Title: NOVEL PROTEASES AND USES THEREOF. Applicant: CARBIOS. The sequence listing filed with the application follows.

SEQUENCE LISTING (28 sequences)

SEQ ID NO: 1 - protein, 276 aa, Actinomadura sp [sequence omitted]

SEQ ID NO: 2 - protein, 81 aa, artificial sequence
  propeptide
APAVPVAMAAAGQGVAGQYIVTLKKGVSVDSTVAKRGIRTQHRFGKVLNGFSAKLTDDQLSKLRTTPGVASIEQDAVITVD

SEQ ID NO: 3 - protein, 22 aa, artificial sequence
  PelB signal peptide
MKYLLPTAAAGLLLLAAQPAMA

SEQ ID NO: 4 - protein, 357 aa, Actinomadura sp.
APAVPVAMAAAGQGVAGQYIVTLKKGVSVDSTVAKRGIRTQHRFGKVLNGFSAKLTDDQLSKLRTTPGVASIEQDAVITVDATQNNPPSWGLDRIDQTNLPLSRSYTYNSTGAGVNAYIIDTGIYTAHSDFGGRATNVYDALGGNGQDCNGHGTHVAGTVGGAAYGVAKAVNLRGVRVLNCSGSGTTSGVIAGMNWVASNHVKPAVANMSLGGGYSSSLNTAANNLASSGVFLAVAAGNETTNACNRSPASAANATTVAASTSTDARASYSNYGSCVHLYAPGSSITSAWLNGGTNTISGTSMATPHVAGTAALYKATYGDASFSTIRSWLVSNATSGVITGNVSGTPNLLLNKRSL

SEQ ID NO: 5 - DNA, 1071 bp, artificial sequnce
  gene encoding non-matured protease
gcccccgctgtccccgtcgccatggccgctgccggccagggtgtcgccggccagtacatcgttactctgaagaagggcgtgtctgttgactctaccgttgctaagcgaggcatccgaacccagcaccgattcggaaaggtcctgaacggattttccgccaagctcaccgacgatcagctgtctaagctccgaaccactcccggcgtcgcctctatcgagcaggacgctgttattaccgtcgatgccactcagaacaaccctccctcctggggtctcgaccgaatcgaccagaccaacctgcctctctctcgatcgtacacctacaactctactggagccggcgtcaacgcttacatcattgacaccggaatttacactgcccactccgatttcggcggtcgagctaccaacgtgtacgacgccctgggaggcaacggtcaggattgcaacggtcacggaacccatgtggccggcactgttggtggagccgcttacggtgtcgccaaggctgtgaacctgcgaggtgtccgagtgctcaactgttccggctctggtaccacttccggagtcatcgctggcatgaactgggtggcctctaaccatgttaagcccgccgtcgctaacatgtccctgggcggtggatactcctcttcgctgaacaccgccgctaacaacctcgcttcctctggagtgttcctggccgttgccgctggcaacgagaccactaacgcctgcaaccgatcgcctgcttccgccgctaacgctaccactgtggccgcttcgacctctactgacgcccgagcttcttactcgaactacggttcttgtgttcacctctacgctcccggatcgtccatcacctctgcctggctgaacggcggtaccaacactatttctggcacctcgatggccactcctcatgttgctggtaccgccgctctctacaaggccacttacggagacgcttccttttctaccattcgatcctggctggtgtctaacgccacctcgggtgtcatcactggtaacgtctctggaactcccaacctgctcctgaacaagcgaagcctg

SEQ ID NO: 6 - protein, 8 aa, artificial sequence
  6xhistidine tag
LEHHHHHH

SEQ ID NO: 7 - DNA, 36 bp, artificial sequence
  PAM S101F forward
gtccgagtgctcaactgtttcggctctggtaccact

SEQ ID NO: 8 - DNA, 36 bp, artificial sequence
  PAM S101L forward
gtccgagtgctcaactgtctgggctctggtaccact

SEQ ID NO: 9 - DNA, 36 bp, artificial sequence
  PAM S101M forward
gtccgagtgctcaactgtatgggctctggtaccact

SEQ ID NO: 10 - DNA, 36 bp, artificial sequence
  PAM S101W forward
gtccgagtgctcaactgttggggctctggtaccact

SEQ ID NO: 11 - DNA, 36 bp, artificial sequence
  PAM S101Y forward
gtccgagtgctcaactgttacggctctggtaccact

SEQ ID NO: 12 - DNA, 36 bp, artificial sequence
  PAM S101 reverse
acagttgagcactcggacacctcgcaggttcacagc

SEQ ID NO: 13 - DNA, 35 bp, artificial sequence
  PAM S103L forward
tgctcaactgttccggcctgggtaccacttccgga

SEQ ID NO: 14 - DNA, 33 bp, artificial sequence
  PAM S103 reverse
gccggaacagttgagcactcggacacctcgcag

SEQ ID NO: 15 - DNA, 35 bp, artificial sequence
  PAM T106I forward
gttccggctctggtaccatctccggagtcatcgct

SEQ ID NO: 16 - DNA, 35 bp, artificial sequence
  PAM T106L forward
gttccggctctggtaccctgtccggagtcatcgct

SEQ ID NO: 17 - DNA, 36 bp, artificial sequence
  PAM T106 reverse
ggtaccagagccggaacagttgagcactcggacacc

SEQ ID NO: 18 - DNA, 34 bp, artificial sequence
  PAM G131I forward
cgctaacatgtccctgatcggtggatactcctct

SEQ ID NO: 19 - DNA, 33 bp, artificial sequence
  PAM G131 reverse
cagggacatgttagcgacggcgggcttaacatg

SEQ ID NO: 20 - DNA, 36 bp, artificial sequence
  PAM G133K forward
ctaacatgtccctgggcggtaagtactcctcttcgc

SEQ ID NO: 21 - DNA, 33 bp, artificial sequence
  PAM G133 reverse
gcccagggacatgttagcgacggcgggcttaac

SEQ ID NO: 22 - DNA, 27 bp, artificial sequence
  PAM_S101F_S103L
gagtgctcaactgtttcggcctgggta

SEQ ID NO: 23 - DNA, 27 bp, artificial sequence
  PAM_S101F_S103L reverse
tcggaagtggtacccaggccgaaacag

SEQ ID NO: 24 - DNA, 30 bp, artificial sequence
  PAM_S101F_S103L_T106I forward
actgtttcggcctgggtaccatctccggag

SEQ ID NO: 25 - DNA, 31 bp, artificial sequence
  PAM_S101F_S103L_T106I reverse
ggagatggtacccaggccgaaacagttgagc

SEQ ID NO: 26 - DNA, 22 bp, artificial sequence
  PAM_T106L bis forward
ggtaccctgtccggagtcatcg

SEQ ID NO: 27 - DNA, 20 bp, artificial sequence
  PAM_S103L_T106L  reverse
tccggacagggtacccaggc

SEQ ID NO: 28 - protein, 386 aa, artificial sequence
  protease
MRRRTLPIAVLAAVPLAMAGALPAGAAPAAPAVPVAMAAAGQGVTGQYIVTLKKGVSVDSTVSKRGIRTQYRFGKVLNGFSAKLTDAQLAKLRTTPGVASIEQDAVIKADATQTNPPSWGIDRIDQTNLPLSNSYTYNSTGAGVNAYIIDTGIYTAHPNFGGRATNVYDALGGNGQDCNGHGTHVAGTVGSTSYGVAKSVNLRGVRVLNCSGSGTTSGVIAGMNWVAGNHVKPAVANMSLGGGYSSSINTAANNLANAGVFLAAAAGNENTNACNRSPASAANATTVAASTSTDARASYSNYGSCVHLYAPGSSITSTWLNGGTNTISGTSMATPHVAGVAALYKATYGDASFSTIRSWLTSNATSGVITGNPSGTPNRLLNKRSL